European Patent Application EP 4 714 494 A2, published March 25, 2026. Title: A MYOSTATIN PATHWAY INHIBITOR IN COMBINATION WITH A GLP-1 PATHWAY ACTIVATOR FOR USE IN TREATING METABOLIC DISORDERS. Applicant: SCHOLAR ROCK, INC. Application EP 25220159.5, filed June 22, 2022. The sequence listing filed with the application follows.

SEQUENCE LISTING (133 sequences)

SEQ ID NO: 1 - protein, 6 aa, synthetic construct
  REGION 1..6: note = Description of Artificial Sequence: Synthetic peptide
SSYGMH

SEQ ID NO: 2 - protein, 10 aa, synthetic construct
  REGION 1..10: note = Description of Artificial Sequence: Synthetic peptide
GFTFSSYGMH

SEQ ID NO: 3 - protein, 10 aa, synthetic construct
  REGION 1..10: note = Description of Artificial Sequence: Synthetic peptide
GFAFSSYGMH

SEQ ID NO: 4 - protein, 17 aa, synthetic construct
  REGION 1..17: note = Description of Artificial Sequence: Synthetic peptide
VISYDGSNKYYADSVKG

SEQ ID NO: 5 - protein, 7 aa, synthetic construct
  REGION 1..7: note = Description of Artificial Sequence: Synthetic peptide
ISYDGSN

SEQ ID NO: 6 - protein, 17 aa, synthetic construct
  REGION 1..17: note = Description of Artificial Sequence: Synthetic peptide
VISYDGSIKYYADSVKG

SEQ ID NO: 7 - protein, 7 aa, synthetic construct
  REGION 1..7: note = Description of Artificial Sequence: Synthetic peptide
ISYDGSI

SEQ ID NO: 8 - protein, 17 aa, synthetic construct
  REGION 1..17: note = Description of Artificial Sequence: Synthetic peptide
VISYDGNNKYYADSVKG

SEQ ID NO: 9 - protein, 7 aa, synthetic construct
  REGION 1..7: note = Description of Artificial Sequence: Synthetic peptide
ISYDGNN

SEQ ID NO: 10 - protein, 17 aa, synthetic construct
  REGION 1..17: note = Description of Artificial Sequence: Synthetic peptide
DLLVRFLEWSHYYGMDV

SEQ ID NO: 11 - protein, 17 aa, synthetic construct
  REGION 1..17: note = Description of Artificial Sequence: Synthetic peptide
DLLVRFLEWSHKYGMDV

SEQ ID NO: 12 - protein, 13 aa, synthetic construct
  REGION 1..13: note = Description of Artificial Sequence: Synthetic peptide
SGSSSNIGSNTVH

SEQ ID NO: 13 - protein, 8 aa, synthetic construct
  REGION 1..8: note = Description of Artificial Sequence: Synthetic peptide
SSNIGSNT

SEQ ID NO: 14 - protein, 13 aa, synthetic construct
  REGION 1..13: note = Description of Artificial Sequence: Synthetic peptide
SGSTSNIGSNTVH

SEQ ID NO: 15 - protein, 8 aa, synthetic construct
  REGION 1..8: note = Description of Artificial Sequence: Synthetic peptide
TSNIGSNT

SEQ ID NO: 16 - protein, 13 aa, synthetic construct
  REGION 1..13: note = Description of Artificial Sequence: Synthetic peptide
SGSSSNIGGNTVH

SEQ ID NO: 17 - skipped

SEQ ID NO: 18 - protein, 16 aa, synthetic construct
  REGION 1..16: note = Description of Artificial Sequence: Synthetic peptide
IISYAGSTYYASWAKG

SEQ ID NO: 19 - protein, 11 aa, synthetic construct
  REGION 1..11: note = Description of Artificial Sequence: Synthetic peptide
  MOD_RES 7: note = Any amino acid
GVPAYSXGGDL

SEQ ID NO: 20 - protein, 13 aa, synthetic construct
  REGION 1..13: note = Description of Artificial Sequence: Synthetic peptide
  MOD_RES 1..2: note = Any amino acid
  MOD_RES 8..9: note = Any amino acid
XXSQSVYXXNWLS

SEQ ID NO: 21 - protein, 7 aa, synthetic construct
  REGION 1..7: note = Description of Artificial Sequence: Synthetic peptide
  MOD_RES 7: note = Any amino acid
WASTLAX

SEQ ID NO: 22 - protein, 10 aa, synthetic construct
  REGION 1..10: note = Description of Artificial Sequence: Synthetic peptide
  MOD_RES 8: note = Any amino acid
AGGYGGGXYA

SEQ ID NO: 23 - protein, 10 aa, synthetic construct
  REGION 1..10: note = Description of Artificial Sequence: Synthetic peptide
AAWDESLNGV

SEQ ID NO: 24 - protein, 126 aa, synthetic construct
  REGION 1..126: note = Description of Artificial Sequence: Synthetic polypeptide
QIQLVQSGGGVVQPGRSLRLSCAASGFTFSSYGMHWVRQAPGKGLEWVAVISYDGSNKYYADSVKGRFTISRDNSKNTLYLQMNSLRAEDTAVYYCARDLLVRFLEWSHYYGMDVWGQGTTVTVSS

SEQ ID NO: 25 - protein, 126 aa, synthetic construct
  REGION 1..126: note = Description of Artificial Sequence: Synthetic polypeptide
QVQLVESGGGVVQPGRSLRLSCAASGFTFSSYGMHWVRQAPGKGLEWVAVISYDGSNKYYADSVKGRFTISRDNSKNTLYLQMNSLRAEDTAVYYCARDLLVRFLEWSHYYGMDVWGQGTTVTVSS

SEQ ID NO: 26 - protein, 126 aa, synthetic construct
  REGION 1..126: note = Description of Artificial Sequence: Synthetic polypeptide
QIQLVQSGGGVVQPGRSLRLSCAASGFAFSSYGMHWVRQAPGKGLEWVAVISYDGSIKYYADSVKGRFTISRDNSKNTLYLQMNSLRAEDTAVYYCARDLLVRFLEWSHKYGMDVWGQGTTVTVSS

SEQ ID NO: 27 - protein, 126 aa, synthetic construct
  REGION 1..126: note = Description of Artificial Sequence: Synthetic polypeptide
QVQLVESGGGVVQPGRSLRLSCAASGFAFSSYGMHWVRQAPGKGLEWVAVISYDGSIKYYADSVKGRFTISRDNSKNTLYLQMNSLRAEDTAVYYCARDLLVRFLEWSHKYGMDVWGQGTTVTVSS

SEQ ID NO: 28 - protein, 126 aa, synthetic construct
  REGION 1..126: note = Description of Artificial Sequence: Synthetic polypeptide
QIQLVQSGGGVVQPGRSLRLSCAASGFAFSSYGMHWVRQAPGKGLEWVAVISYDGNNKYYADSVKGRFTISRDNSKNTLYLQMNSLRAEDTAVYYCARDLLVRFLEWSHKYGMDVWGQGTTVTVSS

SEQ ID NO: 29 - protein, 126 aa, synthetic construct
  REGION 1..126: note = Description of Artificial Sequence: Synthetic polypeptide
QVQLVESGGGVVQPGRSLRLSCAASGFAFSSYGMHWVRQAPGKGLEWVAVISYDGNNKYYADSVKGRFTISRDNSKNTLYLQMNSLRAEDTAVYYCARDLLVRFLEWSHKYGMDVWGQGTTVTVSS

SEQ ID NO: 30 - protein, 109 aa, synthetic construct
  REGION 1..109: note = Description of Artificial Sequence: Synthetic polypeptide
QPVLTQPPSASGTPGQRVTISCSGSSSNIGSNTVHWYQQLPGTAPKLLIYSDNQRPSGVPDRFSGSKSGTSASLVISGLQSDDEADYYCAAWDDSLNGVFGGGTKLTVL

SEQ ID NO: 31 - protein, 109 aa, synthetic construct
  REGION 1..109: note = Description of Artificial Sequence: Synthetic polypeptide
QSVLTQPPSASGTPGQRVTISCSGSSSNIGSNTVHWYQQLPGTAPKLLIYSDNQRPSGVPDRFSGSKSGTSASLAISGLQSEDEADYYCAAWDDSLNGVFGGGTKLTVL

SEQ ID NO: 32 - protein, 109 aa, synthetic construct
  REGION 1..109: note = Description of Artificial Sequence: Synthetic polypeptide
QPVLTQPPSASGTPGQRVTISCSGSTSNIGSNTVHWYQQLPGTAPKLLIYSDDQRPSGVPDRFSGSKSGTSASLVISGLQSDDEADYYCAAWDESLNGVFGGGTKLTVL

SEQ ID NO: 33 - protein, 109 aa, synthetic construct
  REGION 1..109: note = Description of Artificial Sequence: Synthetic polypeptide
QSVLTQPPSASGTPGQRVTISCSGSTSNIGSNTVHWYQQLPGTAPKLLIYSDDQRPSGVPDRFSGSKSGTSASLAISGLQSEDEADYYCAAWDESLNGVFGGGTKLTVL

SEQ ID NO: 34 - protein, 109 aa, synthetic construct
  REGION 1..109: note = Description of Artificial Sequence: Synthetic polypeptide
QPVLTQPPSASGTPGQRVTISCSGSSSNIGGNTVHWYQQLPGTAPKLLIYSDDQRPSGVPDRFSGSKSGTSASLVISGLQSDDEADYYCAAWDESLNGVFGGGTKLTVL

SEQ ID NO: 35 - protein, 109 aa, synthetic construct
  REGION 1..109: note = Description of Artificial Sequence: Synthetic polypeptide
QSVLTQPPSASGTPGQRVTISCSGSSSNIGGNTVHWYQQLPGTAPKLLIYSDDQRPSGVPDRFSGSKSGTSASLAISGLQSEDEADYYCAAWDESLNGVFGGGTKLTVL

SEQ ID NO: 36 - protein, 98 aa, synthetic construct
  REGION 1..98: note = Description of Artificial Sequence: Synthetic polypeptide
QVQLVESGGGVVQPGRSLRLSCAASGFTFSSYGMHWVRQAPGKGLEWVAVISYDGSNKYYADSVKGRFTISRDNSKNTLYLQMNSLRAEDTAVYYCAR

SEQ ID NO: 37 - protein, 98 aa, synthetic construct
  REGION 1..98: note = Description of Artificial Sequence: Synthetic polypeptide
QSVLTQPPSASGTPGQRVTISCSGSSSNIGSNTVNWYQQLPGTAPKLLIYSNNQRPSGVPDRFSGSKSGTSASLAISGLQSEDEADYYCAAWDDSLNG

SEQ ID NO: 38 - DNA, 378 bp, synthetic construct
  misc_feature 1..378: note = Description of Artificial Sequence: Synthetic polynucleotide
  source 1..378: mol_type = other DNA
cagatccagctggtgcagtctgggggaggcgtggtccagcctgggaggtccctgagactctcctgtgcagcgtctggattcaccttcagtagctatggcatgcactgggtccgccaggctccaggcaaggggctggagtgggtggcagttatatcatatgatggaagtaataaatactatgcagactccgtgaagggccgattcaccatctccagagacaattccaagaacacgctgtatctgcaaatgaacagcctgagagccgaggacacggctgtgtattactgtgcgagagatctcctggtgcgatttttggagtggtcgcactactacggtatggacgtctggggccaagggaccacggtcaccgtctcctca

SEQ ID NO: 39 - DNA, 378 bp, synthetic construct
  misc_feature 1..378: note = Description of Artificial Sequence: Synthetic polynucleotide
  source 1..378: mol_type = other DNA
caggtgcagctggtggagtctgggggaggcgtggtccagcctgggaggtccctgagactctcctgtgcagcgtctggattcaccttcagtagctatggcatgcactgggtccgccaggctccaggcaaggggctggagtgggtggcagttatatcatatgatggaagtaataaatactatgcagactccgtgaagggccgattcaccatctccagagacaattccaagaacacgctgtatctgcaaatgaacagcctgagagccgaggacacggctgtgtattactgtgcgagagatctcctggtgcgatttttggagtggtcgcactactacggtatggacgtctggggccaagggaccacggtcaccgtctcctca

SEQ ID NO: 40 - DNA, 378 bp, synthetic construct
  misc_feature 1..378: note = Description of Artificial Sequence: Synthetic polynucleotide
  source 1..378: mol_type = other DNA
cagatccagctggtgcagtctgggggaggcgtggtccagcctgggaggtccctgagactctcctgtgcagcgtctggattcgccttcagtagctatggcatgcactgggtccgccaggctccaggcaaggggctggagtgggtggcagttatatcatatgatggaagtatcaaatactatgcagactccgtgaagggccgattcaccatctccagagacaattccaagaacacgctgtatctgcaaatgaacagcctgagagccgaggacacggctgtgtattactgtgcgagagatctcctggtgcgatttttggagtggtcgcacaagtacggtatggacgtctggggccaagggaccacggtcaccgtctcctca

SEQ ID NO: 41 - DNA, 378 bp, synthetic construct
  misc_feature 1..378: note = Description of Artificial Sequence: Synthetic polynucleotide
  source 1..378: mol_type = other DNA
caggtgcagctggtggagtctgggggaggcgtggtccagcctgggaggtccctgagactctcctgtgcagcgtctggattcgccttcagtagctatggcatgcactgggtccgccaggctccaggcaaggggctggagtgggtggcagttatatcatatgatggaagtatcaaatactatgcagactccgtgaagggccgattcaccatctccagagacaattccaagaacacgctgtatctgcaaatgaacagcctgagagccgaggacacggctgtgtattactgtgcgagagatctcctggtgcgatttttggagtggtcgcacaagtacggtatggacgtctggggccaagggaccacggtcaccgtctcctca

SEQ ID NO: 42 - DNA, 378 bp, synthetic construct
  misc_feature 1..378: note = Description of Artificial Sequence: Synthetic polynucleotide
  source 1..378: mol_type = other DNA
cagatccagctggtgcagtctgggggaggcgtggtccagcctgggaggtccctgagactctcctgtgcagcgtctggattcgccttcagtagctatggcatgcactgggtccgccaggctccaggcaaggggctggagtgggtggcagttatatcatatgatggaaataataaatactatgcagactccgtgaagggccgattcaccatctccagagacaattccaagaacacgctgtatctgcaaatgaacagcctgagagccgaggacacggctgtgtattactgtgcgagagatctcctggtgcgatttttggagtggtcgcacaagtacggtatggacgtctggggccaagggaccacggtcaccgtctcctca

SEQ ID NO: 43 - DNA, 378 bp, synthetic construct
  misc_feature 1..378: note = Description of Artificial Sequence: Synthetic polynucleotide
  source 1..378: mol_type = other DNA
caggtgcagctggtggagtctgggggaggcgtggtccagcctgggaggtccctgagactctcctgtgcagcgtctggattcgccttcagtagctatggcatgcactgggtccgccaggctccaggcaaggggctggagtgggtggcagttatatcatatgatggaaataataaatactatgcagactccgtgaagggccgattcaccatctccagagacaattccaagaacacgctgtatctgcaaatgaacagcctgagagccgaggacacggctgtgtattactgtgcgagagatctcctggtgcgatttttggagtggtcgcacaagtacggtatggacgtctggggccaagggaccacggtcaccgtctcctca

SEQ ID NO: 44 - DNA, 327 bp, synthetic construct
  misc_feature 1..327: note = Description of Artificial Sequence: Synthetic polynucleotide
  source 1..327: mol_type = other DNA
cagcctgtgctgactcagccaccctcagcgtctgggacccccgggcagagggtcaccatctcttgttctggaagcagctccaacatcggaagtaatactgtccactggtaccagcaactcccaggaacggcccccaaactcctcatctatagtgataatcagcgcccctcaggggtccctgaccgattctctggctccaagtctggcacctcagcctccctggtcatcagtgggctccagtctgacgatgaggctgattattactgtgcagcatgggatgacagcctgaatggggtgttcggcggagggaccaagctgaccgtccta

SEQ ID NO: 45 - DNA, 327 bp, synthetic construct
  misc_feature 1..327: note = Description of Artificial Sequence: Synthetic polynucleotide
  source 1..327: mol_type = other DNA
cagtctgtgctgactcagccaccctcagcgtctgggacccccgggcagagggtcaccatctcttgttctggaagcagctccaacatcggaagtaatactgtccactggtaccagcaactcccaggaacggcccccaaactcctcatctatagtgataatcagcgcccctcaggggtccctgaccgattctctggctccaagtctggcacctcagcctccctggccatcagtgggctccagtctgaggatgaggctgattattactgtgcagcatgggatgacagcctgaatggggtgttcggcggagggaccaagctgaccgtccta

SEQ ID NO: 46 - DNA, 327 bp, synthetic construct
  misc_feature 1..327: note = Description of Artificial Sequence: Synthetic polynucleotide
  source 1..327: mol_type = other DNA
cagcctgtgctgactcagccaccctcagcgtctgggacccccgggcagagggtcaccatctcttgttctggaagcacctccaacatcggaagtaatactgtccactggtaccagcaactcccaggaacggcccccaaactcctcatctatagtgatgatcagcgcccctcaggggtccctgaccgattctctggctccaagtctggcacctcagcctccctggtcatcagtgggctccagtctgacgatgaggctgattattactgtgcagcatgggatgagagcctgaatggggtgttcggcggagggaccaagctgaccgtccta

SEQ ID NO: 47 - DNA, 327 bp, synthetic construct
  misc_feature 1..327: note = Description of Artificial Sequence: Synthetic polynucleotide
  source 1..327: mol_type = other DNA
cagtctgtgctgactcagccaccctcagcgtctgggacccccgggcagagggtcaccatctcttgttctggaagcacctccaacatcggaagtaatactgtccactggtaccagcaactcccaggaacggcccccaaactcctcatctatagtgatgatcagcgcccctcaggggtccctgaccgattctctggctccaagtctggcacctcagcctccctggccatcagtgggctccagtctgaggatgaggctgattattactgtgcagcatgggatgagagcctgaatggggtgttcggcggagggaccaagctgaccgtccta

SEQ ID NO: 48 - DNA, 327 bp, synthetic construct
  misc_feature 1..327: note = Description of Artificial Sequence: Synthetic polynucleotide
  source 1..327: mol_type = other DNA
cagcctgtgctgactcagccaccctcagcgtctgggacccccgggcagagggtcaccatctcttgttctggaagcagctccaacatcggaggaaatactgtccactggtaccagcaactcccaggaacggcccccaaactcctcatctatagtgatgatcagcgcccctcaggggtccctgaccgattctctggctccaagtctggcacctcagcctccctggtcatcagtgggctccagtctgacgatgaggctgattattactgtgcagcatgggatgagagcctgaatggggtgttcggcggagggaccaagctgaccgtccta

SEQ ID NO: 49 - DNA, 327 bp, synthetic construct
  misc_feature 1..327: note = Description of Artificial Sequence: Synthetic polynucleotide
  source 1..327: mol_type = other DNA
cagtctgtgctgactcagccaccctcagcgtctgggacccccgggcagagggtcaccatctcttgttctggaagcagctccaacatcggaggaaatactgtccactggtaccagcaactcccaggaacggcccccaaactcctcatctatagtgatgatcagcgcccctcaggggtccctgaccgattctctggctccaagtctggcacctcagcctccctggccatcagtgggctccagtctgaggatgaggctgattattactgtgcagcatgggatgagagcctgaatggggtgttcggcggagggaccaagctgaccgtccta

SEQ ID NO: 50 - protein, 452 aa, synthetic construct
  REGION 1..452: note = Description of Artificial Sequence: Synthetic polypeptide
QVQLVESGGGVVQPGRSLRLSCAASGFTFSSYGMHWVRQAPGKGLEWVAVISYDGSNKYYADSVKGRFTISRDNSKNTLYLQMNSLRAEDTAVYYCARDLLVRFLEWSHYYGMDVWGQGTTVTVSSASTKGPSVFPLAPCSRSTSESTAALGCLVKDYFPEPVTVSWNSGALTSGVHTFPAVLQSSGLYSLSSVVTVPSSSLGTKTYTCNVDHKPSNTKVDKRVESKYGPPCPPCPAPEFLGGPSVFLFPPKPKDTLMISRTPEVTCVVVDVSQEDPEVQFNWYVDGVEVHNAKTKPREEQFNSTYRVVSVLTVLHQDWLNGKEYKCKVSNKGLPSSIEKTISKAKGQPREPQVYTLPPSQEEMTKNQVSLTCLVKGFYPSDIAVEWESNGQPENNYKTTPPVLDSDGSFFLYSRLTVDKSRWQEGNVFSCSVMHEALHNHYTQKSLSLSLG

SEQ ID NO: 51 - protein, 215 aa, synthetic construct
  REGION 1..215: note = Description of Artificial Sequence: Synthetic polypeptide
QSVLTQPPSASGTPGQRVTISCSGSSSNIGSNTVHWYQQLPGTAPKLLIYSDNQRPSGVPDRFSGSKSGTSASLAISGLQSEDEADYYCAAWDDSLNGVFGGGTKLTVLGQPKAAPSVTLFPPSSEELQANKATLVCLISDFYPGAVTVAWKADSSPVKAGVETTTPSKQSNNKYAASSYLSLTPEQWKSHRSYSCQVTHEGSTVEKTVAPTECS

SEQ ID NO: 52 - protein, 352 aa, Homo sapiens [sequence omitted]

SEQ ID NO: 53 - protein, 352 aa, Rattus sp.
NEDSEREANVEKEGLCNACAWRQNTRYSRIEAIKIQILSKLRLETAPNISKDAIRQLLPRAPPLRELIDQYDVQRDDSSDGSLEDDDYHATTETIITMPTESDFLMQADGKPKCCFFKFSSKIQYNKVVKAQLWIYLRAVKTPTTVFVQILRLIKPMKDGTRYTGIRSLKLDMSPGTGIWQSIDVKTVLQNWLKQPESNLGIEIKALDENGHDLAVTFPGPGEDGLNPFLEVKVTDTPKRSRRDFGLDCDEHSTESRCCRYPLTVDFEAFGWDWIIAPKRYKANYCSGECEFVFLQKYPHTHLVHQANPRGSAGPCCTPTKMSPINMLYFNGKEQIIYGKIPAMVVDRCGCS

SEQ ID NO: 54 - protein, 352 aa, Mus sp.
NEGSEREENVEKEGLCNACAWRQNTRYSRIEAIKIQILSKLRLETAPNISKDAIRQLLPRAPPLRELIDQYDVQRDDSSDGSLEDDDYHATTETIITMPTESDFLMQADGKPKCCFFKFSSKIQYNKVVKAQLWIYLRPVKTPTTVFVQILRLIKPMKDGTRYTGIRSLKLDMSPGTGIWQSIDVKTVLQNWLKQPESNLGIEIKALDENGHDLAVTFPGPGEDGLNPFLEVKVTDTPKRSRRDFGLDCDEHSTESRCCRYPLTVDFEAFGWDWIIAPKRYKANYCSGECEFVFLQKYPHTHLVHQANPRGSAGPCCTPTKMSPINMLYFNGKEQIIYGKIPAMVVDRCGCS

SEQ ID NO: 55 - protein, 277 aa, Macaca fascicularis
NENSEQKENVEKEGLCNACTWRQNTKSSRIEAIKIQILSKLRLETAPNISKDAIRQLLPKAPPLRELIDQYDVQRDDSSDGSLEDDDYHATTETIITMPTESDFLMQVDGKPKCCFFKFSSKIQYNKVVKAQLWIYLRPVETPTTVFVQILRLIKPMKDGTRYTGIRSLKLDMNPGTGIWQSIDVKTVLQNWLKQPESNLGIEIKALDENGHDLAVTFPGPGEDGLNPFLEVKVTDTPKRSRRDFGLDCDEHSTESRCCRYPLTVDFEAFGWDWIIA

SEQ ID NO: 56 - protein, 109 aa, unidentified
  REGION 1..109: note = Description of Unknown: Mature myostatin sequence
DFGLDCDEHSTESRCCRYPLTVDFEAFGWDWIIAPKRYKANYCSGECEFVFLQKYPHTHLVHQANPRGSAGPCCTPTKMSPINMLYFNGKEQIIYGKIPAMVVDRCGCS

SEQ ID NO: 57 - protein, 24 aa, unidentified
  REGION 1..24: note = Description of Unknown: Antibody binding epitope sequence
FVQILRLIKPMKDGTRYTGIRSLK

SEQ ID NO: 58 - protein, 5 aa, synthetic construct
  REGION 1..5: note = Description of Artificial Sequence: Synthetic peptide
CPPCP

SEQ ID NO: 59 - protein, 8 aa, synthetic construct
  REGION 1..8: note = Description of Artificial Sequence: Synthetic peptide
SSNIGGNT

SEQ ID NO: 60 - protein, 7 aa, synthetic construct
  REGION 1..7: note = Description of Artificial Sequence: Synthetic peptide
SDNQRPS

SEQ ID NO: 61 - skipped

SEQ ID NO: 62 - protein, 33 aa, unidentified
  REGION 1..33: note = Description of Unknown: Antibody binding sequence
PKAPPLRELIDQYDVQRDDSSDGSLEDDDYHAT

SEQ ID NO: 63 - protein, 34 aa, unidentified
  REGION 1..34: note = Description of Unknown: Antibody binding sequence
GLNPFLEVKVTDTPKRSRRDFGLDCDEHSTESRC

SEQ ID NO: 64 - skipped

SEQ ID NO: 65 - protein, 10 aa, synthetic construct
  REGION 1..10: note = Description of Artificial Sequence: Synthetic peptide
AAWDDSLNGV

SEQ ID NO: 66 - protein, 5 aa, synthetic construct
  REGION 1..5: note = Description of Artificial Sequence: Synthetic peptide
SYDIS

SEQ ID NO: 67 - protein, 11 aa, synthetic construct
  REGION 1..11: note = Description of Artificial Sequence: Synthetic peptide
GVPAYSTGGDL

SEQ ID NO: 68 - protein, 13 aa, synthetic construct
  REGION 1..13: note = Description of Artificial Sequence: Synthetic peptide
QSSQSVYDNNWLS

SEQ ID NO: 69 - protein, 7 aa, synthetic construct
  REGION 1..7: note = Description of Artificial Sequence: Synthetic peptide
WASTLAS

SEQ ID NO: 70 - protein, 10 aa, synthetic construct
  REGION 1..10: note = Description of Artificial Sequence: Synthetic peptide
AGGYGGGLYA

SEQ ID NO: 71 - protein, 17 aa, synthetic construct
  REGION 1..17: note = Description of Artificial Sequence: Synthetic peptide
ESLIRFLEDPQQGGMDV

SEQ ID NO: 72 - protein, 10 aa, synthetic construct
  REGION 1..10: note = Description of Artificial Sequence: Synthetic peptide
NSWTRSNNYI

SEQ ID NO: 73 - protein, 126 aa, synthetic construct
  REGION 1..126: note = Description of Artificial Sequence: Synthetic polypeptide
QVQLQQSGAEVKKPGASVKVSCKASGYTFTSYYMHWVRQAPGQGLEWMGIINPSGGSTSYAQKFQGRVTMTRDTSTSTVYMELSSLRSEDTAVYYCARESLIRFLEDPQQGGMDVWGQGTTVTVSS

SEQ ID NO: 74 - protein, 121 aa, synthetic construct
  REGION 1..121: note = Description of Artificial Sequence: Synthetic polypeptide
QSALTQPASVSGSPGQSLTISCTGTSSDIGGYNYVSWYQQHPGKAPKLIIYDVTDRPSGVSGRFSGSKSGNTASLTISGLQTEDEAEYFCNSWTRSNNYIFGGGTKLTVLGQPKAAPSVTL

SEQ ID NO: 75 - protein, 273 aa, synthetic construct
  REGION 1..273: note = Description of Artificial Sequence: Synthetic polypeptide
QVQLQQSGAEVKKPGASVKVSCKASGYTFTSYYMHWVRQAPGQGLEWMGIINPSGGSTSYAQKFQGRVTMTRDTSTSTVYMELSSLRSEDTAVYYCARESLIRFLEDPQQGGMDVWGQGTTVTVSSGSASAPTLGGGGSGGGGSAAAQSALTQPASVSGSPGQSLTISCTGTSSDIGGYNYVSWYQQHPGKAPKLIIYDVTDRPSGVSGRFSGSKSGNTASLTISGLQTEDEAEYFCNSWTRSNNYIFGGGTKLTVLGQPKAAPSVTLFPPSS

SEQ ID NO: 76 - protein, 13 aa, synthetic construct
  REGION 1..13: note = Description of Artificial Sequence: Synthetic peptide
DRYSSSWGGGFDY

SEQ ID NO: 77 - protein, 10 aa, synthetic construct
  REGION 1..10: note = Description of Artificial Sequence: Synthetic peptide
QSYDASSLWV

SEQ ID NO: 78 - protein, 122 aa, synthetic construct
  REGION 1..122: note = Description of Artificial Sequence: Synthetic polypeptide
EVQLVQSGGGVVQSGRSLRLSCVASGFSFSNYGMHWVRQAPGKGLEWLAFIWYDGSNKWYADSVKGRFTISRDNSKNALYLQMNSLRAEDTAVYYCARDRYSSSWGGGFDYWGQGTVLTVSS

SEQ ID NO: 79 - protein, 122 aa, synthetic construct
  REGION 1..122: note = Description of Artificial Sequence: Synthetic polypeptide
NFMLTQPHSVSESPGRTVTIPCSGRGGSIASDSVQWYQQRPGSAPTTIIYEDNQRPSGVPDRFSGSVDSSSNSASLTISGLRTEDEADYYCQSYDASSLWVFGGKTKLTVLGQPKAAPSVTL

SEQ ID NO: 80 - protein, 275 aa, synthetic construct
  REGION 1..275: note = Description of Artificial Sequence: Synthetic polypeptide
EVQLVQSGGGVVQSGRSLRLSCVASGFSFSNYGMHWVRQAPGKGLEWLAFIWYDGSNKWYADSVKGRFTISRDNSKNALYLQMNSLRAEDTAVYYCARDRYSSSWGGGFDYWGQGTVLTVSSGSASAPTLGGGGSGGGGSAAANFMLTQPHSVSESPGRTVTIPCSGRGGSIASDSVQWYQQRPGSAPTTIIYEDNQRPSGVPDRFSGSVDSSSNSASLTISGLRTEDEADYYCQSYDASSLWVFGGKTKLTVLGQPKAAPSVTLFPPSSKASGA

SEQ ID NO: 81 - protein, 10 aa, synthetic construct
  REGION 1..10: note = Description of Artificial Sequence: Synthetic peptide
DRHSLGDFDY

SEQ ID NO: 82 - protein, 9 aa, synthetic construct
  REGION 1..9: note = Description of Artificial Sequence: Synthetic peptide
QAWDSTTVV

SEQ ID NO: 83 - protein, 121 aa, synthetic construct
  REGION 1..121: note = Description of Artificial Sequence: Synthetic polypeptide
QLQLQQSGGGLVKPGGSLRLSCAASGFTFSSYSMNWVRQAPGKGLEWVSSISSSSSYIYYADSVKGRFTISRDNAKNSLYLQMNSLRAEDTAVYYCVRDRHSLGDFDYWGQGTLVTVSSGS

SEQ ID NO: 84 - protein, 121 aa, synthetic construct
  REGION 1..121: note = Description of Artificial Sequence: Synthetic polypeptide
SSELTQPSVSVSPGQTATITCSGDKLGDKYASWYQQKPGQSPVLVIYQDTKRPSGIPARFSGSNSGNTATLTISGTQAMDEAAYYCQAWDSTTVVFGGGTKLTVLGQPKAAPSVTLFPPSS

SEQ ID NO: 85 - protein, 201 aa, synthetic construct
  REGION 1..201: note = Description of Artificial Sequence: Synthetic polypeptide
QLQLQQSGGGLVKPGGSLRLSCAASGFTFSSYSMNWVRQAPGKGLEWVSSISSSSSYIYYADSVKGRFTISRDNAKNSLYLQMNSLRAEDTAVYYCVRDRHSLGDFDYWGQGTLVTVSSGSASAPTLGGGGSGGGGSAAASSELTQPPSVSVSPGQTATITCSGDKLGDKYASWYQQKPGQSPVLVIYQDTKRPSGIPARF

SEQ ID NO: 86 - protein, 18 aa, synthetic construct
  REGION 1..18: note = Description of Artificial Sequence: Synthetic peptide
HGLMDDSSGYYLSNAFDI

SEQ ID NO: 87 - protein, 11 aa, synthetic construct
  REGION 1..11: note = Description of Artificial Sequence: Synthetic peptide
ATWDDSLTGVV

SEQ ID NO: 88 - protein, 129 aa, synthetic construct
  REGION 1..129: note = Description of Artificial Sequence: Synthetic polypeptide
QVQLVQSGAEVKKPGSSVKVSCKASGGTFSSYAISWVRQAPGQGLEWMGGIIPIFGTANYAQKFQGRVTITADESTSTAYMELSSLRSEDTAVYYCANHGLMDDSSGYYLSNAFDIWGQGTMVTVSSGS

SEQ ID NO: 89 - protein, 126 aa, synthetic construct
  REGION 1..126: note = Description of Artificial Sequence: Synthetic polypeptide
QPVLTQPPSASGTPGQRVTISCSGSSSNIGSNTVEWYQQLPGTAPKLLIHSNNQRPSGVPDRFSGSRSGTSASLAISGLQSEDEADYFCATWDDSLTGVVFGGGTTLTVLGQPKAAPSVTLFPPSS

SEQ ID NO: 90 - protein, 274 aa, synthetic construct
  REGION 1..274: note = Description of Artificial Sequence: Synthetic polypeptide
QVQLVQSGAEVKKPGSSVKVSCKASGGTFSSYAISWVRQAPGQGLEWMGGIIPIFGTANYAQKFQGRVTITADESTSTAYMELSSLRSEDTAVYYCANHGLMDDSSGYYLSNAFDIWGQGTMVTVSSGSASAPTLGGGGSGGGGSAAAQPVLTQPPSASGTPGQRVTISCSGSSSNIGSNTVEWYQQLPGTAPKLLIHSNNQRPSGVPDRFSGSRSGTSASLAISGLQSEDEADYFCATWDDSLTGVVFGGGTTLTVLGQPKAAPSVTLFPPSS

SEQ ID NO: 91 - protein, 12 aa, synthetic construct
  REGION 1..12: note = Description of Artificial Sequence: Synthetic peptide
VGTAAAGDAFDI

SEQ ID NO: 92 - protein, 11 aa, synthetic construct
  REGION 1..11: note = Description of Artificial Sequence: Synthetic peptide
AAWDDSLSGWV

SEQ ID NO: 93 - protein, 123 aa, synthetic construct
  REGION 1..123: note = Description of Artificial Sequence: Synthetic polypeptide
QVQLVQSGGGLIQPGGSLRLSCAASGFTVSSYSMNWVRQAPGKGLEWVSYISSSGSTIYYADSVKGRFTISRDNAKNSLYLQMNSLRAEDTALYYCAKVGTAAAGDAFDIWGQGTMVTVSSGS

SEQ ID NO: 94 - protein, 126 aa, synthetic construct
  REGION 1..126: note = Description of Artificial Sequence: Synthetic polypeptide
QPVLTQPPSASGTPGQRVTISCFGSSSNIGSNYVYWYQQLPGTAPKLLIYRNNQRPSGVPDRFSGSKSGTSASLAISGLRSEDEADYYCAAWDDSLSGWVFGGGTKLTVLGQPKAAPSVTLFPPSS

SEQ ID NO: 95 - protein, 268 aa, synthetic construct
  REGION 1..268: note = Description of Artificial Sequence: Synthetic polypeptide
QVQLVQSGGGLIQPGGSLRLSCAASGFTVSSYSMNWVRQAPGKGLEWVSYISSSGSTIYYADSVKGRFTISRDNAKNSLYLQMNSLRAEDTALYYCAKVGTAAAGDAFDIWGQGTMVTVSSGSASAPTLGGGGSGGGGSAAAQPVLTQPPSASGTPGQRVTISCFGSSSNIGSNYVYWYQQLPGTAPKLLIYRNNQRPSGVPDRFSGSKSGTSASLAISGLRSEDEADYYCAAWDDSLSGWVFGGGTKLTVLGQPKAAPSVTLFPPSS

SEQ ID NO: 96 - protein, 18 aa, synthetic construct
  REGION 1..18: note = Description of Artificial Sequence: Synthetic peptide
VGFYDYVWGSYPYDAFDI

SEQ ID NO: 97 - protein, 9 aa, synthetic construct
  REGION 1..9: note = Description of Artificial Sequence: Synthetic peptide
QQYGTSPLT

SEQ ID NO: 98 - protein, 127 aa, synthetic construct
  REGION 1..127: note = Description of Artificial Sequence: Synthetic polypeptide
QIQLVQSGAEVKKPGASVKVSCKASGYTFTSYGISWVRQAPGQGLEWMGWISAYNGNTNYAQKLQGRVTMTTDTSTSTAYMELSSLRSEDTAVYYCARVGFYDYVWGSYPYDAFDIWGQGTMVTVSS

SEQ ID NO: 99 - protein, 108 aa, synthetic construct
  REGION 1..108: note = Description of Artificial Sequence: Synthetic polypeptide
EIVMTQSPGTLSLSPGERATLSCRASQSVSSNYLAWYQQKPGQAPRLLIYDASNRATGIPARFSGSGSGTDFTLTISSLEPEDFALYYCQQYGTSPLTFGGGTKLEIK

SEQ ID NO: 100 - protein, 265 aa, synthetic construct
  REGION 1..265: note = Description of Artificial Sequence: Synthetic polypeptide
QIQLVQSGAEVKKPGASVKVSCKASGYTFTSYGISWVRQAPGQGLEWMGWISAYNGNTNYAQKLQGRVTMTTDTSTSTAYMELSSLRSEDTAVYYCARVGFYDYVWGSYPYDAFDIWGQGTMVTVSSGSASAPTLGGGGSGGGGSAAAEIVMTQSPGTLSLSPGERATLSCRASQSVSSNYLAWYQQKPGQAPRLLIYDASNRATGIPARFSGSGSGTDFTLTISSLEPEDFALYYCQQYGTSPLTFGGGTKLEIKRTVAAPSVF

SEQ ID NO: 101 - protein, 14 aa, synthetic construct
  REGION 1..14: note = Description of Artificial Sequence: Synthetic peptide
DTSNGGYSSSSFDY

SEQ ID NO: 102 - protein, 10 aa, synthetic construct
  REGION 1..10: note = Description of Artificial Sequence: Synthetic peptide
SSYTSSSTLV

SEQ ID NO: 103 - protein, 123 aa, synthetic construct
  REGION 1..123: note = Description of Artificial Sequence: Synthetic polypeptide
EVQLVQSGGGLVQPGRSLRLSCAASGFTFDDYAMHWVRQAPGKGLEWVSGISWNSGSIGYADSVKGRFTISRDNAKNSLYLQMNSLRAEDTALYYCAKDTSNGGYSSSSFDYWGQGTLVTVSS

SEQ ID NO: 104 - protein, 110 aa, synthetic construct
  REGION 1..110: note = Description of Artificial Sequence: Synthetic polypeptide
QSALTQPASVSGSPGQSITISCTGTSSDVGGYNYVSWYQQHPGTAPKLMIYDVSYRPSGVSNRFSGSKSGNTASLTISGLQAEDEADYYCSSYTSSSTLVFGTGTKVTVL

SEQ ID NO: 105 - protein, 270 aa, synthetic construct
  REGION 1..270: note = Description of Artificial Sequence: Synthetic polypeptide
EVQLVQSGGGLVQPGRSLRLSCAASGFTFDDYAMHWVRQAPGKGLEWVSGISWNSGSIGYADSVKGRFTISRDNAKNSLYLQMNSLRAEDTALYYCAKDTSNGGYSSSSFDYWGQGTLVTVSSGSASAPTLGGGGSGGGGSAAAQSALTQPASVSGSPGQSITISCTGTSSDVGGYNYVSWYQQHPGTAPKLMIYDVSYRPSGVSNRFSGSKSGNTASLTISGLQAEDEADYYCSSYTSSSTLVFGTGTKVTVLGQPKANPTVTLFPPSS

SEQ ID NO: 106 - protein, 15 aa, synthetic construct
  REGION 1..15: note = Description of Artificial Sequence: Synthetic peptide
LVYGGYDEPGYYFDY

SEQ ID NO: 107 - protein, 11 aa, synthetic construct
  REGION 1..11: note = Description of Artificial Sequence: Synthetic peptide
AAWDDSLNGWV

SEQ ID NO: 108 - protein, 124 aa, synthetic construct
  REGION 1..124: note = Description of Artificial Sequence: Synthetic polypeptide
EVQLLESRAEVKKPGESLKISCKGSGYSFTSYWIGWVRQMPGKGPEWMGIIYPGDSDTRYSPSFQGQVTISADKSISTAYLQWSSLKASDTAMYYCARLVYGGYDEPGYYFDYWGQGTLVTVSS

SEQ ID NO: 109 - protein, 110 aa, synthetic construct
  REGION 1..110: note = Description of Artificial Sequence: Synthetic polypeptide
QSVLTQPPSASGTPGQRVTISCSGSSSNIRSNTVNWYQQLPGTAPKLLIYSNNQRPSGVPDRFSGSKSGTSASLAISGLQSEDEADYYCAAWDDSLNGWVFGGGTKLTVL

SEQ ID NO: 110 - protein, 276 aa, synthetic construct
  REGION 1..276: note = Description of Artificial Sequence: Synthetic polypeptide
EVQLLESRAEVKKPGESLKISCKGSGYSFTSYWIGWVRQMPGKGPEWMGIIYPGDSDTRYSPSFQGQVTISADKSISTAYLQWSSLKASDTAMYYCARLVYGGYDEPGYYFDYWGQGTLVTVSSGSASAPTLGGGGSGGGGSAAAQSVLTQPPSASGTPGQRVTISCSGSSSNIRSNTVNWYQQLPGTAPKLLIYSNNQRPSGVPDRFSGSKSGTSASLAISGLQSEDEADYYCAAWDDSLNGWVFGGGTKLTVLGQPKAAPSVTLFPPSSKASGA

SEQ ID NO: 111 - protein, 14 aa, synthetic construct
  REGION 1..14: note = Description of Artificial Sequence: Synthetic peptide
VDGLEYSSGHNFDY

SEQ ID NO: 112 - protein, 10 aa, synthetic construct
  REGION 1..10: note = Description of Artificial Sequence: Synthetic peptide
SSYAGSYTWV

SEQ ID NO: 113 - protein, 123 aa, synthetic construct
  REGION 1..123: note = Description of Artificial Sequence: Synthetic polypeptide
EVQLVQSGGGLVQPGRSLRLSCAASGFTFDDYAMHWVRQAPGKGLEWVSGISWNSGSIGYADSVKGRFTISRDNSKNTLYLQMNSLRAEDTAVYYCAKVDGLEYSSGHNFDYWGQGTLVTVSS

SEQ ID NO: 114 - protein, 110 aa, synthetic construct
  REGION 1..110: note = Description of Artificial Sequence: Synthetic polypeptide
QSALTQPPSVSGSPGQSVTISCTGSSSDVGYYDHVSWYQHHPGRAPKVIIYDVTKRPSGVPDRFSGSKSGNTASLTISGLQAEDEADYYCSSYAGSYTWVFGGGTELTVL

SEQ ID NO: 115 - protein, 270 aa, synthetic construct
  REGION 1..270: note = Description of Artificial Sequence: Synthetic polypeptide
EVQLVQSGGGLVQPGRSLRLSCAASGFTFDDYAMHWVRQAPGKGLEWVSGISWNSGSIGYADSVKGRFTISRDNSKNTLYLQMNSLRAEDTAVYYCAKVDGLEYSSGHNFDYWGQGTLVTVSSGSASAPTLGGGGSGGGGSAAAQSALTQPPSVSGSPGQSVTISCTGSSSDVGYYDHVSWYQHHPGRAPKVIIYDVTKRPSGVPDRFSGSKSGNTASLTISGLQAEDEADYYCSSYAGSYTWVFGGGTELTVLGQPKAAPSVTLFPPSS

SEQ ID NO: 116 - protein, 7 aa, unidentified
  REGION 1..7: note = Description of Unknown: GLP-1 analog sequence
EGTFTSD

SEQ ID NO: 117 - protein, 9 aa, unidentified
  REGION 1..9: note = Description of Unknown: GLP-1 analog sequence
  MOD_RES 2..3: note = Any amino acid
  MOD_RES 5: note = Any amino acid
  MOD_RES 8: note = Any amino acid
HXXGXFTXD

SEQ ID NO: 118 - protein, 6 aa, unidentified
  REGION 1..6: note = Description of Unknown: Antibody binding epitope sequence
KALDEN

SEQ ID NO: 119 - protein, 5 aa, synthetic construct
  REGION 1..5: note = Description of Artificial Sequence: Synthetic peptide
HTDIS

SEQ ID NO: 120 - protein, 11 aa, synthetic construct
  REGION 1..11: note = Description of Artificial Sequence: Synthetic peptide
GVPAYSHGGDL

SEQ ID NO: 121 - protein, 7 aa, synthetic construct
  REGION 1..7: note = Description of Artificial Sequence: Synthetic peptide
WASTLAY

SEQ ID NO: 122 - protein, 10 aa, synthetic construct
  REGION 1..10: note = Description of Artificial Sequence: Synthetic peptide
AGGYGGGRYA

SEQ ID NO: 123 - protein, 5 aa, synthetic construct
  REGION 1..5: note = Description of Artificial Sequence: Synthetic peptide
HDDIS

SEQ ID NO: 124 - protein, 13 aa, synthetic construct
  REGION 1..13: note = Description of Artificial Sequence: Synthetic peptide
TTSQSVYHENWLS

SEQ ID NO: 125 - protein, 116 aa, synthetic construct
  REGION 1..116: note = Description of Artificial Sequence: Synthetic polypeptide
QSLEESGGRLVTPGGSLTVTCRVSGIDLSSYDISWVRQAPGKGLEWIGIISYAGSTYYASWAKGRFTISKTSTTVDLKMTSLTTEDTATYFCARGVPAYSTGGDLWGPGTLVTVSS

SEQ ID NO: 126 - protein, 119 aa, synthetic construct
  REGION 1..119: note = Description of Artificial Sequence: Synthetic polypeptide
QVTLKESGPVLVKPTETLTLTCTVSGIDLSSYDISWVRQAPGKGLEWVGIISYAGSTYYASWAKGRLTISKDTSKNQVVLTMTNMDPVDTATYYCARGVPAYSTGGDLWGQGTLVTVSS

SEQ ID NO: 127 - protein, 119 aa, synthetic construct
  REGION 1..119: note = Description of Artificial Sequence: Synthetic polypeptide
QVTLKESGPVLVKPTETLTLTCTVSGIDLSHTDISWVRQAPGKGLEWVGIISYAGSTYYASWAKGRLTISKDTSKNQVVLTMTNMDPVDTATYYCARGVPAYSHGGDLWGQGTLVTVSS

SEQ ID NO: 128 - protein, 119 aa, synthetic construct
  REGION 1..119: note = Description of Artificial Sequence: Synthetic polypeptide
QVQLVESGGGLVQPGGSLRLSCAVSGIDLSHDDISWVRQAPGKGLEWVSIISYAGSTYYASWAKGRLTISKDTSKNQVVLTMTNMDPVDTATYYCARGVPAYSHGGDLWGQGTLVTVSS

SEQ ID NO: 129 - protein, 110 aa, synthetic construct
  REGION 1..110: note = Description of Artificial Sequence: Synthetic polypeptide
AQVLTQTASSVSAAVGGTVTINCQSSQSVYDNNWLSWFQQKPGQPPKLLIYWASTLASGVPSRFKGSGSGTQFTLTISDLECDDAATYYCAGGYGGGLYAFGGGTKVEIK

SEQ ID NO: 130 - protein, 110 aa, synthetic construct
  REGION 1..110: note = Description of Artificial Sequence: Synthetic polypeptide
DIVMTQSPATLSLSPGERATLSCTTSQSVYHENWLSWFQQKPGQPPKLLIYWASTLAYGVPSRFSGSGSGTDFTLTISSLQPEDAATYYCAGGYGGGRYAFGQGTKVEIK

SEQ ID NO: 131 - protein, 7 aa, synthetic construct
  REGION 1..7: note = Description of Artificial Sequence: Synthetic peptide
SDDQRPS

SEQ ID NO: 132 - protein, 110 aa, synthetic construct
  REGION 1..110: note = Description of Artificial Sequence: Synthetic polypeptide
DIVMTQSPATLSLSPGERATLSCQSSQSVYDNNWLSWFQQKPGQPPKLLIYWASTLASGVPSRFSGSGSGTDFTLTISSLQPEDAATYYCAGGYGGGLYAFGQGTKVEIK

SEQ ID NO: 133 - protein, 110 aa, synthetic construct
  REGION 1..110: note = Description of Artificial Sequence: Synthetic polypeptide
DIVMTQSPATLSLSPGERATLSCTSSQSVYHNNWLSWFQQKPGQPPKLLIYWASTLAYGVPSRFSGSGSGTDFTLTISSLQPEDAATYYCAGGYGGGRYAFGQGTKVEIK